European Patent Application EP 4 261 230 A1, published October 18, 2023. Title: RECOMBINANT HUMAN SERUM ALBUMIN-COLLAGEN BINDING DOMAIN FUSION PROTEIN FOR TUMOR-SPECIFIC TARGETING MATRIX, AND USE THEREOF. Applicant: Huatong Forturn (China) Co., Ltd. Beijing Bio-Fortune Ltd. Huatong Forturn Biopharmaceutical (Shandong) Co., Ltd. The sequence listing filed with the application follows.

SEQUENCE LISTING (8 sequences)

SEQ ID NO: 1 - protein, 790 aa, Artificial Sequence
  Amino acid sequence of a recombinant fusion protein
CSGEGLQIPTLSPAPDCSQPLDVILLLDGSSSFPASYFDEMKSFAKAFISKANIGPRLTQVSVLQYGSITTIDVPWNVVPEKAHLLSLVDVMQREGGPSQIGDALGFAVRYLTSEMHGARPGASKAVVILVTDVSVDSVDAAADAARSNRVTVFPIGIGDRYDAAQLRILAGPAGDSNVVKLQRIEDLPTMVTLGNSFLHKLCSGDAHKSEVAHRFKDLGEENFKALVLIAFAQYLQQCPFEDHVKLVNEVTEFAKTCVADESAENCDKSLHTLFGDKLCTVATLRETYGEMADCCAKQEPERNECFLQHKDDNPNLPRLVRPEVDVMCTAFHDNEETFLKKYLYEIARRHPYFYAPELLFFAKRYKAAFTECCQAADKAACLLPKLDELRDEGKASSAKQRLKCASLQKFGERAFKAWAVARLSQRFPKAEFAEVSKLVTDLTKVHTECCHGDLLECADDRADLAKYICENQDSISSKLKECCEKPLLEKSHCIAEVENDEMPADLPSLAADFVESKDVCKNYAEAKDVFLGMFLYEYARRHPDYSVVLLLRLAKTYETTLEKCCAAADPHECYAKVFDEFKPLVEEPQNLIKQNCELFEQLGEYKFQNALLVRYTKKVPEVSTPTLVEVSRNLGKVGSKCCKHPEAKRMPCAEDYLSVVLNQLCVLHEKTPVSDRVTKCCTESLVNRRPCFSALEVDETYVPKEFNAETFTFHADICTLSEKERQIKKQTALVELVKHKPKATKEQLKAVMDDFAAFVEKCCKADDKETCFAEEGKKLVAASQAALGL

SEQ ID NO: 2 - DNA, 2376 bp, Artificial Sequence
  Nucleotide sequence encoding a recombinant fusion protein
tgttctggtgaaggtttgcaaattccaactttgtctccagctccagattgttctcaaccattggatgttattttgttgttggatggttcttcttcttttccagcttcttactttgatgaaatgaagtcttttgctaaggcttttatttctaaggctaacattggtccaagattgactcaagtttctgttttgcaatacggttctattactactattgatgttccatggaacgttgttccagaaaaggctcatttgttgtctttggttgatgttatgcaaagagaaggtggtccatctcaaattggtgatgctttgggttttgctgttagatacttgacttctgaaatgcatggtgctagaccaggtgcttctaaggctgttgttattttggttactgatgtttctgttgattctgttgatgctgctgctgatgctgctagatctaacagagttactgtttttccaattggtattggtgatagatacgatgctgctcaattgagaattttggctggtccagctggtgattctaacgttgttaagttgcaaagaattgaagatttgccaactatggttactttgggtaactcttttttgcataagttgtgttctggtgatgctcacaagagtgaggttgctcatcggtttaaagatttgggagaagaaaatttcaaagccttggtgttgattgcctttgctcagtatcttcagcagtgtccatttgaagatcatgtaaaattagtgaatgaagtaactgaatttgcaaaaacatgtgttgctgatgagtcagctgaaaattgtgacaaatcacttcataccctttttggagacaaattatgcacagttgcaactcttcgtgaaacctatggtgaaatggctgactgctgtgcaaaacaagaacctgagagaaatgaatgcttcttgcaacacaaagatgacaacccaaacctcccccgattggtgagaccagaggttgatgtgatgtgcactgcttttcatgacaatgaagagacatttttgaaaaaatacttatatgaaattgccagaagacatccttacttttatgccccggaactccttttctttgctaaaaggtataaagctgcttttacagaatgttgccaagctgctgataaagctgcctgcctgttgccaaagctcgatgaacttcgggatgaagggaaggcttcgtctgccaaacagagactcaagtgtgccagtctccaaaaatttggagaaagagctttcaaagcatgggcagtagctcgcctgagccagagatttcccaaagctgagtttgcagaagtttccaagttagtgacagatcttaccaaagtccacacggaatgctgccatggagatctgcttgaatgtgctgatgacagggcggaccttgccaagtatatctgtgaaaatcaagattcgatctccagtaaactgaaggaatgctgtgaaaaacctctgttggaaaaatcccactgcattgccgaagtggaaaatgatgagatgcctgctgacttgccttcattagctgctgattttgttgaaagtaaggatgtttgcaaaaactatgctgaggcaaaggatgtcttcctgggcatgtttttgtatgaatatgcaagaaggcatcctgattactctgtcgtgctgctgctgagacttgccaagacatatgaaaccactctagagaagtgctgtgccgctgcagatcctcatgaatgctatgccaaagtgttcgatgaatttaaacctcttgtggaagagcctcagaatttaatcaaacaaaattgtgagctttttgagcagcttggagagtacaaattccagaatgcgctattagttcgttacaccaagaaagtaccccaagtgtcaactccaactcttgtagaggtctcaagaaacctaggaaaagtgggcagcaaatgttgtaaacatcctgaagcaaaaagaatgccctgtgcagaagactatctatccgtggtcctgaaccagttatgtgtgttgcatgagaaaacgccagtaagtgacagagtcaccaaatgctgcacagaatccttggtgaacaggcgaccatgcttttcagctctggaagtcgatgaaacatacgttcccaaagagtttaatgctgaaacattcaccttccatgcagatatatgcacactttctgagaaggagagacaaatcaagaaacaaactgcacttgttgagcttgtgaaacacaagcccaaggcaacaaaagagcaactgaaagctgttatggatgatttcgcagcttttgtagagaagtgctgcaaggctgacgataaggagacctgctttgccgaggagggtaaaaaacttgttgctgcaagtcaagctgccttaggcttatgataa

SEQ ID NO: 3 - protein, 798 aa, Artificial Sequence
  Amino acid sequence of a recombinant fusion protein 2
DAHKSEVAHRFKDLGEENFKALVLIAFAQYLQQCPFEDHVKLVNEVTEFAKTCVADESAENCDKSLHTLFGDKLCTVATLRETYGEMADCCAKQEPERNECFLQHKDDNPNLPRLVRPEVDVMCTAFHDNEETFLKKYLYEIARRHPYFYAPELLFFAKRYKAAFTECCQAADKAACLLPKLDELRDEGKASSAKQRLKCASLQKFGERAFKAWAVARLSQRFPKAEFAEVSKLVTDLTKVHTECCHGDLLECADDRADLAKYICENQDSISSKLKECCEKPLLEKSHCIAEVENDEMPADLPSLAADFVESKDVCKNYAEAKDVFLGMFLYEYARRHPDYSVVLLLRLAKTYETTLEKCCAAADPHECYAKVFDEFKPLVEEPQNLIKQNCELFEQLGEYKFQNALLVRYTKKVPQVSTPTLVEVSRNLGKVGSKCCKHPEAKRMPCAEDYLSVVLNQLCVLHEKTPVSDRVTKCCTESLVNRRPCFSALEVDETYVPKEFNAETFTFHADICTLSEKERQIKKQTALVELVKHKPKATKEQLKAVMDDFAAFVEKCCKADDKETCFAEEGKKLVAASQAALGLGGGSGGGSCSGEGLQIPTLSPAPDCSQPLDVILLLDGSSSFPASYFDEMKSFAKAFISKANIGPRLTQVSVLQYGSITTIDVPWNVVPEKAHLLSLVDVMQREGGPSQIGDALGFAVRYLTSEMHGARPGASKAVVILVTDVSVDSVDAAADAARSNRVTVFPIGIGDRYDAAQLRILAGPAGDSNVVKLQRIEDLPTMVTLGNSFLHKLCSG

SEQ ID NO: 4 - DNA, 2472 bp, Artificial Sequence
  Nucleotide sequence encoding a recombinant fusion protein 2
atgaagtgggtaacctttatttcccttctttttctctttagctcggcttattccaggggtgtgtttcgtcgagatgcacacaagagtgaggttgctcatcggtttaaagatttgggagaagaaaatttcaaagccttggtgttgattgcctttgctcagtatcttcagcagtgtccatttgaagatcatgtaaaattagtgaatgaagtaactgaatttgcaaaaacatgtgttgctgatgagtcagctgaaaattgtgacaaatcacttcataccctttttggagacaaattatgcacagttgcaactcttcgtgaaacctatggtgaaatggctgactgctgtgcaaaacaagaacctgagagaaatgaatgcttcttgcaacacaaagatgacaacccaaacctcccccgattggtgagaccagaggttgatgtgatgtgcactgcttttcatgacaatgaagagacatttttgaaaaaatacttatatgaaattgccagaagacatccttacttttatgccccggaactccttttctttgctaaaaggtataaagctgcttttacagaatgttgccaagctgctgataaagctgcctgcctgttgccaaagctcgatgaacttcgggatgaagggaaggcttcgtctgccaaacagagactcaagtgtgccagtctccaaaaatttggagaaagagctttcaaagcatgggcagtagctcgcctgagccagagatttcccaaagctgagtttgcagaagtttccaagttagtgacagatcttaccaaagtccacacggaatgctgccatggagatctgcttgaatgtgctgatgacagggcggaccttgccaagtatatctgtgaaaatcaagattcgatctccagtaaactgaaggaatgctgtgaaaaacctctgttggaaaaatcccactgcattgccgaagtggaaaatgatgagatgcctgctgacttgccttcattagctgctgattttgttgaaagtaaggatgtttgcaaaaactatgctgaggcaaaggatgtcttcctgggcatgtttttgtatgaatatgcaagaaggcatcctgattactctgtcgtgctgctgctgagacttgccaagacatatgaaaccactctagagaagtgctgtgccgctgcagatcctcatgaatgctatgccaaagtgttcgatgaatttaaacctcttgtggaagagcctcagaatttaatcaaacaaaattgtgagctttttgagcagcttggagagtacaaattccagaatgcgctattagttcgttacaccaagaaagtaccccaagtgtcaactccaactcttgtagaggtctcaagaaacctaggaaaagtgggcagcaaatgttgtaaacatcctgaagcaaaaagaatgccctgtgcagaagactatctatccgtggtcctgaaccagttatgtgtgttgcatgagaaaacgccagtaagtgacagagtcaccaaatgctgcacagaatccttggtgaacaggcgaccatgcttttcagctctggaagtcgatgaaacatacgttcccaaagagtttaatgctgaaacattcaccttccatgcagatatatgcacactttctgagaaggagagacaaatcaagaaacaaactgcacttgttgagcttgtgaaacacaagcccaaggcaacaaaagagcaactgaaagctgttatggatgatttcgcagcttttgtagagaagtgctgcaaggctgacgataaggagacctgctttgccgaggagggtaaaaaacttgttgctgcaagtcaagctgccttaggcttaggtggtggttctggtggtggttcttgttctggtgaaggtttgcaaattccaactttgtctccagctccagattgttctcaaccattggatgttattttgttgttggatggttcttcttcttttccagcttcttactttgatgaaatgaagtcttttgctaaggcttttatttctaaggctaacattggtccaagattgactcaagtttctgttttgcaatacggttctattactactattgatgttccatggaacgttgttccagaaaaggctcatttgttgtctttggttgatgttatgcaaagagaaggtggtccatctcaaattggtgatgctttgggttttgctgttagatacttgacttctgaaatgcatggtgctagaccaggtgcttctaaggctgttgttattttggttactgatgtttctgttgattctgttgatgctgctgctgatgctgctagatctaacagagttactgtttttccaattggtattggtgatagatacgatgctgctcaattgagaattttggctggtccagctggtgattctaacgttgttaagttgcaaagaattgaagatttgccaactatggttactttgggtaactcttttttgcataagttgtgttctggttgataa

SEQ ID NO: 5 - DNA, 30 bp, Artificial Sequence
  oligonucleotide primer 1
gaattcatgaagtgggtaacctttatttcc

SEQ ID NO: 6 - DNA, 33 bp, Artificial Sequence
  oligonucleotide primer 2
gaattcttataagcctaaggcagcttgacttgc

SEQ ID NO: 7 - DNA, 19 bp, Artificial Sequence
  P1
ctggttccaattgacaagc

SEQ ID NO: 8 - DNA, 19 bp, Artificial Sequence
  P9
gactcatcagcaacacatg